European Patent Specification EP 4 305 044 B1, published February 18, 2026. Title: 3'3' CYCLIC DINUCLEOTIDES CONTAINING ISONUCLEOTIDIC UNITS. Applicant: Ustav organicke chemie a biochemie AV CR, v. v. i. The sequence listing filed with the application follows.

SEQUENCE LISTING (11 sequences)

SEQ ID NO: 1 - DNA, 75 bp, artificial
  synthetic oligonucleotide
aaagatcttggaaagtgaaaccttggaaaacgaaactggacaaagggaaactgcagaaactgaaacaaagcttaa

SEQ ID NO: 2 - DNA, 75 bp, artificial
  synthetic oligonucleotide
ttaagctttgtttcagtttctgcagtttccctttgtccagtttcgttttccaaggtttcactttccaagatcttt

SEQ ID NO: 3 - DNA, 20 bp, artificial
  primer
tgcttgctcaactctacgtc

SEQ ID NO: 4 - DNA, 20 bp, artificial
  primer
gtggtttgtccaaactcatc

SEQ ID NO: 5 - DNA, 31 bp, artificial
  primer
gtgggatccgccccagctgagatctctgcag

SEQ ID NO: 6 - DNA, 38 bp, artificial
  primer
tatgcggccgcctattacacagtaacctcttccttttc

SEQ ID NO: 7 - DNA, 330 bp, artificial
  DNA sequence of 8-His-SUMO
atgtcgcatcaccatcatcatcaccaccatgggatgtcggactcagaagtcaatcaagaagctaagccagaggtcaagccagaagtcaagcctgagactcacatcaatttaaaggtgtccgatggatcttcagagatcttcttcaagatcaaaaagaccactcctttaagaaggctgatggaagcgttcgctaaaagacagggtaaggaaatggactccttaagattcttgtacgacggtattagaattcaagctgatcagacccctgaagatttggacatggaggataacgatattattgaggctcaccgcgaacagattggtggatcc

SEQ ID NO: 8 - protein, 110 aa, artificial
  Amino acid sequence of 8-His-SUMO
MSHHHHHHHHGMSDSEVNQEAKPEVKPEVKPETHINLKVSDGSSEIFFKIKKTTPLRRLMEAFAKRQGKEMDSLRFLYDGIRIQADQTPEDLDMEDNDIIEAHREQIGGS

SEQ ID NO: 9 - protein, 204 aa, artificial
  Amino acid sequence of truncated WT STING
APAEISAVCEKGNFNVAHGLAWSYYIGYLRLILPELQARIRTYNQHYNNLLRGAVSQRLYILLPLDCGVPDNLSMADPNIRFLDKLPQQTGDRAGIKDRVYSNSIYELLENGQRAGTCVLEYATPLQTLFAMSQYSQAGFSREDRLEQAKLFCRTLEDILADAPESQNNCRLIAYQEPADDSSFSLSQEVLRHLRQEEKEEVTV

SEQ ID NO: 10 - protein, 204 aa, artificial
  Amino acid sequence of truncated AQ STING
APAEISAVCEKGNFNVAHGLAWSYYIGYLRLILPELQARIRTYNQHYNNLLRGAVSQRLYILLPLDCGVPDNLSMADPNIRFLDKLPQQTADRAGIKDRVYSNSIYELLENGQRAGTCVLEYATPLQTLFAMSQYSQAGFSREDRLEQAKLFCQTLEDILADAPESQNNCRLIAYQEPADDSSFSLSQEVLRHLRQEEKEEVTV

SEQ ID NO: 11 - protein, 392 aa, artificial
  Murine cGAS amino acid sequence including pelB leader and His-tag
MKYLLPTAAAGLLLLAAQPAMAMPDKLKKVLDKLRLKRKDISEAAETVNKVVERLLRRMQKRESEFKGVEQLNTGSYYEHVKISAPNEFDVMFKLEVPRIELQEYYETGAFYLVKFKRIPRGNPLSHFLEGEVLSATKMLSKFRKIIKEEVKEIKDIDVSVEKEKPGSPAVTLLIRNPEEISVDIILALESKGSWPISTKEGLPIQGWLGTKVRTNLRREPFYLVPKNAKDGNSFQGETWRLSFSHTEKYILNNHGIEKTCCESSGAKCCRKECLKLMKYLLEQLKKEFQELDAFCSYHVKTAIFHMWTQDPQDSQWDPRNLSSCFDKLLAFFLECLRTEKLDHYFIPKFNLFSQELIDRKSKEFLSKKIEYERNNGFPIFDKLLEHHHHHH